European Patent Application EP 4 806 993 A1, published September 16, 2026. Title: 신규한 바실러스 서브틸리스 BM107 균주 및 이의 용도. Applicant: 주식회사 바이오미. Application WO. The sequence listing filed with the application follows.

SEQUENCE LISTING (2 sequences)

SEQ ID NO: 1 - DNA, 633 bp, Bacillus subtilis
  source 1..633: mol_type = genomic DNA
gtgaaaaaagtacttatggcattcattatttgtttatcgctgattctatctgttttagccgctccgccgtctggcgcaaaagctgagtcagtacataatcctgtcgttcttgttcatggaataagtggtgcatcatacaactttttcgctattaaaaactacttaatttctcaaggctggcaaagcaacaaactgtacgcaattgatttttatgataaaacaggaaacaacctaaataacggcccgcagcttgcttcatatgttgaccgtgttttaaaagagactggggcaaaaaaagtagatattgtggctcatagtatgggaggcgccaatacgctgtactatattaaatatttaggcgggggcaataagattcaaaatgtcgtaacgcttggaggggctaatggtttagtgtcatcaaccgcgctgccgggcacagaccctaatcaaaagatcctctatacatctatttacagtctcaatgatcaaattgtcatcaatagcttgtctcggttacaaggagcgcgaaacatccagctttatggcatcggtcatattggcttgctttctaatagccaagtgaacggctatatcaaagaagggctgaatggcggaggcctcaatacaaattaa

SEQ ID NO: 2 - protein, 210 aa, Bacillus subtilis
MKKVLMAFIICLSLILSVLAAPPSGAKAESVHNPVVLVHGISGASYNFFAIKNYLISQGWQSNKLYAIDFYDKTGNNLNNGPQLASYVDRVLKETGAKKVDIVAHSMGGANTLYYIKYLGGGNKIQNVVTLGGANGLVSSTALPGTDPNQKILYTSIYSLNDQIVINSLSRLQGARNIQLYGIGHIGLLSNSQVNGYIKEGLNGGGLNTN